European Patent Application EP 4 744 656 A1, published May 20, 2026. Title: USE OF DIVALENT METAL LACTATE IN PREPARATION OF PRODUCTS THAT PROMOTE TISSUE GROWTH AND REPAIR. Applicant: CHANGCHUN SINOBIOMATERIALS CO., LTD. The sequence listing filed with the application follows.

SEQUENCE LISTING (4 sequences)

SEQ ID NO: 1 - DNA, 20 bp, synthetic construct
  source 1..20: mol_type = other DNA
gagcttggaacggtacgata

SEQ ID NO: 2 - DNA, 20 bp, synthetic construct
  source 1..20: mol_type = other DNA
ccgtaccagagcgagatgac

SEQ ID NO: 3 - DNA, 21 bp, synthetic construct
  source 1..21: mol_type = other DNA
ggagtaccctgatgagatcga

SEQ ID NO: 4 - DNA, 23 bp, synthetic construct
  source 1..23: mol_type = other DNA
ctttggtctgcattcacatttgt